European Patent Application EP 4 506 450 A1, published February 12, 2025. Title: MODIFIED ESTERASE. Applicant: 天野エンザイム株式会社. The sequence listing filed with the application follows.

SEQUENCE LISTING (30 sequences)

SEQ ID NO: 1 - protein, 375 aa, synthetic construct
  REGION 1..375: note = a matured form of a standard esterase (quintuple mutant)
VDAQTIAPGFESVAELFGRFLSEDREYSAQLAAYHRGVKVLDISGGPHRRPDSVTGVFSCSKGVSGLVIALLVQDGFLDLDAEVVKYWPEFGAEGKATITVAQLLSHQAGLLGVEGGLTLAEYNNSELAAAKLAQMRPLWKPGTAFGYHALTIGVFMEELCRRITGSTLQEIYEQRIRSVTGAHFFLGLPESEEPRYATLRWAADPSQPWIDPASHFGLSFDSAVGDILDLPNLREVRAAGLSSAAGVASAEGMARVYAAALTGLAANGDRAAVAPLLSEETIQTVTAEQVFGIDRVLGETSCFGTVFMKSHARSPYGSYRAFGHVGGSASLGFADPVYELAFGYVPQQAEPGGAGCRNLELSAAVRKAVTELAQ

SEQ ID NO: 2 - protein, 383 aa, synthetic construct
  REGION 1..383: note = a full-length form of a standard esterase (quintuple mutant)
MTMITPSLVDAQTIAPGFESVAELFGRFLSEDREYSAQLAAYHRGVKVLDISGGPHRRPDSVTGVFSCSKGVSGLVIALLVQDGFLDLDAEVVKYWPEFGAEGKATITVAQLLSHQAGLLGVEGGLTLAEYNNSELAAAKLAQMRPLWKPGTAFGYHALTIGVFMEELCRRITGSTLQEIYEQRIRSVTGAHFFLGLPESEEPRYATLRWAADPSQPWIDPASHFGLSFDSAVGDILDLPNLREVRAAGLSSAAGVASAEGMARVYAAALTGLAANGDRAAVAPLLSEETIQTVTAEQVFGIDRVLGETSCFGTVFMKSHARSPYGSYRAFGHVGGSASLGFADPVYELAFGYVPQQAEPGGAGCRNLELSAAVRKAVTELAQ

SEQ ID NO: 3 - protein, 375 aa, Arthrobacter globiformis
VDAQTIAPGFESVAELFGRFLSEDREYSAQLAAYHRGVKVLDISGGPHRRPDSVTGVFSCSKGVSGLVIALLVQDGFLDLDAEVVKYWPEFGAEGKATITVAQLLSHQAGLLGVEGGLTLAEYNNSELAAAKLAQMRPLWKPGTAFGYHALTIGVFMEELCRRITGSTLQEIYEQRIRSVTGAHFFLGLPESEEPRYATLRWAADPSQPWIDPASHFGLSANSAVGDILDLPNLREVRAAGLSSAAGVASAEGMARVYAAALTGLAANGDRAAVAPLLSEETIQTVTAEQVFGIDRVFGETSCFGTVFMKSHARSPYGSYRAFGHDGASASLGFADPVYELAFGYVPQQAEPGGAGCRNLELSAAVRKAVTELAQ

SEQ ID NO: 4 - protein, 383 aa, Arthrobacter globiformis
MTMITPSLVDAQTIAPGFESVAELFGRFLSEDREYSAQLAAYHRGVKVLDISGGPHRRPDSVTGVFSCSKGVSGLVIALLVQDGFLDLDAEVVKYWPEFGAEGKATITVAQLLSHQAGLLGVEGGLTLAEYNNSELAAAKLAQMRPLWKPGTAFGYHALTIGVFMEELCRRITGSTLQEIYEQRIRSVTGAHFFLGLPESEEPRYATLRWAADPSQPWIDPASHFGLSANSAVGDILDLPNLREVRAAGLSSAAGVASAEGMARVYAAALTGLAANGDRAAVAPLLSEETIQTVTAEQVFGIDRVFGETSCFGTVFMKSHARSPYGSYRAFGHDGASASLGFADPVYELAFGYVPQQAEPGGAGCRNLELSAAVRKAVTELAQ

SEQ ID NO: 5 - protein, 375 aa, synthetic construct
  REGION 1..375: note = L151F mutant of SEQ ID NO:1
VDAQTIAPGFESVAELFGRFLSEDREYSAQLAAYHRGVKVLDISGGPHRRPDSVTGVFSCSKGVSGLVIALLVQDGFLDLDAEVVKYWPEFGAEGKATITVAQLLSHQAGLLGVEGGLTLAEYNNSELAAAKLAQMRPLWKPGTAFGYHAFTIGVFMEELCRRITGSTLQEIYEQRIRSVTGAHFFLGLPESEEPRYATLRWAADPSQPWIDPASHFGLSFDSAVGDILDLPNLREVRAAGLSSAAGVASAEGMARVYAAALTGLAANGDRAAVAPLLSEETIQTVTAEQVFGIDRVLGETSCFGTVFMKSHARSPYGSYRAFGHVGGSASLGFADPVYELAFGYVPQQAEPGGAGCRNLELSAAVRKAVTELAQ

SEQ ID NO: 6 - protein, 375 aa, synthetic construct
  REGION 1..375: note = L242M mutant of SEQ ID NO:1
VDAQTIAPGFESVAELFGRFLSEDREYSAQLAAYHRGVKVLDISGGPHRRPDSVTGVFSCSKGVSGLVIALLVQDGFLDLDAEVVKYWPEFGAEGKATITVAQLLSHQAGLLGVEGGLTLAEYNNSELAAAKLAQMRPLWKPGTAFGYHALTIGVFMEELCRRITGSTLQEIYEQRIRSVTGAHFFLGLPESEEPRYATLRWAADPSQPWIDPASHFGLSFDSAVGDILDLPNLREVRAAGMSSAAGVASAEGMARVYAAALTGLAANGDRAAVAPLLSEETIQTVTAEQVFGIDRVLGETSCFGTVFMKSHARSPYGSYRAFGHVGGSASLGFADPVYELAFGYVPQQAEPGGAGCRNLELSAAVRKAVTELAQ

SEQ ID NO: 7 - protein, 375 aa, synthetic construct
  REGION 1..375: note = S329N mutant of SEQ ID NO:1
VDAQTIAPGFESVAELFGRFLSEDREYSAQLAAYHRGVKVLDISGGPHRRPDSVTGVFSCSKGVSGLVIALLVQDGFLDLDAEVVKYWPEFGAEGKATITVAQLLSHQAGLLGVEGGLTLAEYNNSELAAAKLAQMRPLWKPGTAFGYHALTIGVFMEELCRRITGSTLQEIYEQRIRSVTGAHFFLGLPESEEPRYATLRWAADPSQPWIDPASHFGLSFDSAVGDILDLPNLREVRAAGLSSAAGVASAEGMARVYAAALTGLAANGDRAAVAPLLSEETIQTVTAEQVFGIDRVLGETSCFGTVFMKSHARSPYGSYRAFGHVGGNASLGFADPVYELAFGYVPQQAEPGGAGCRNLELSAAVRKAVTELAQ

SEQ ID NO: 8 - protein, 375 aa, synthetic construct
  REGION 1..375: note = L200F mutant of SEQ ID NO:1
VDAQTIAPGFESVAELFGRFLSEDREYSAQLAAYHRGVKVLDISGGPHRRPDSVTGVFSCSKGVSGLVIALLVQDGFLDLDAEVVKYWPEFGAEGKATITVAQLLSHQAGLLGVEGGLTLAEYNNSELAAAKLAQMRPLWKPGTAFGYHALTIGVFMEELCRRITGSTLQEIYEQRIRSVTGAHFFLGLPESEEPRYATFRWAADPSQPWIDPASHFGLSFDSAVGDILDLPNLREVRAAGLSSAAGVASAEGMARVYAAALTGLAANGDRAAVAPLLSEETIQTVTAEQVFGIDRVLGETSCFGTVFMKSHARSPYGSYRAFGHVGGSASLGFADPVYELAFGYVPQQAEPGGAGCRNLELSAAVRKAVTELAQ

SEQ ID NO: 9 - protein, 375 aa, synthetic construct
  REGION 1..375: note = L151F/L242M mutant of SEQ ID NO:1
VDAQTIAPGFESVAELFGRFLSEDREYSAQLAAYHRGVKVLDISGGPHRRPDSVTGVFSCSKGVSGLVIALLVQDGFLDLDAEVVKYWPEFGAEGKATITVAQLLSHQAGLLGVEGGLTLAEYNNSELAAAKLAQMRPLWKPGTAFGYHAFTIGVFMEELCRRITGSTLQEIYEQRIRSVTGAHFFLGLPESEEPRYATLRWAADPSQPWIDPASHFGLSFDSAVGDILDLPNLREVRAAGMSSAAGVASAEGMARVYAAALTGLAANGDRAAVAPLLSEETIQTVTAEQVFGIDRVLGETSCFGTVFMKSHARSPYGSYRAFGHVGGSASLGFADPVYELAFGYVPQQAEPGGAGCRNLELSAAVRKAVTELAQ

SEQ ID NO: 10 - protein, 375 aa, synthetic construct
  REGION 1..375: note = L151F/L242M/S329N mutant of SEQ ID NO:1
VDAQTIAPGFESVAELFGRFLSEDREYSAQLAAYHRGVKVLDISGGPHRRPDSVTGVFSCSKGVSGLVIALLVQDGFLDLDAEVVKYWPEFGAEGKATITVAQLLSHQAGLLGVEGGLTLAEYNNSELAAAKLAQMRPLWKPGTAFGYHAFTIGVFMEELCRRITGSTLQEIYEQRIRSVTGAHFFLGLPESEEPRYATLRWAADPSQPWIDPASHFGLSFDSAVGDILDLPNLREVRAAGMSSAAGVASAEGMARVYAAALTGLAANGDRAAVAPLLSEETIQTVTAEQVFGIDRVLGETSCFGTVFMKSHARSPYGSYRAFGHVGGNASLGFADPVYELAFGYVPQQAEPGGAGCRNLELSAAVRKAVTELAQ

SEQ ID NO: 11 - protein, 375 aa, synthetic construct
  REGION 1..375: note = L151F/L242M/L200F mutant of SEQ ID NO:1
VDAQTIAPGFESVAELFGRFLSEDREYSAQLAAYHRGVKVLDISGGPHRRPDSVTGVFSCSKGVSGLVIALLVQDGFLDLDAEVVKYWPEFGAEGKATITVAQLLSHQAGLLGVEGGLTLAEYNNSELAAAKLAQMRPLWKPGTAFGYHAFTIGVFMEELCRRITGSTLQEIYEQRIRSVTGAHFFLGLPESEEPRYATFRWAADPSQPWIDPASHFGLSFDSAVGDILDLPNLREVRAAGMSSAAGVASAEGMARVYAAALTGLAANGDRAAVAPLLSEETIQTVTAEQVFGIDRVLGETSCFGTVFMKSHARSPYGSYRAFGHVGGSASLGFADPVYELAFGYVPQQAEPGGAGCRNLELSAAVRKAVTELAQ

SEQ ID NO: 12 - protein, 375 aa, synthetic construct
  REGION 1..375: note = L151F/L242M/L200F/S329N mutant of SEQ ID NO:1
VDAQTIAPGFESVAELFGRFLSEDREYSAQLAAYHRGVKVLDISGGPHRRPDSVTGVFSCSKGVSGLVIALLVQDGFLDLDAEVVKYWPEFGAEGKATITVAQLLSHQAGLLGVEGGLTLAEYNNSELAAAKLAQMRPLWKPGTAFGYHAFTIGVFMEELCRRITGSTLQEIYEQRIRSVTGAHFFLGLPESEEPRYATFRWAADPSQPWIDPASHFGLSFDSAVGDILDLPNLREVRAAGMSSAAGVASAEGMARVYAAALTGLAANGDRAAVAPLLSEETIQTVTAEQVFGIDRVLGETSCFGTVFMKSHARSPYGSYRAFGHVGGNASLGFADPVYELAFGYVPQQAEPGGAGCRNLELSAAVRKAVTELAQ

SEQ ID NO: 13 - DNA, 1128 bp, synthetic construct
  misc_feature 1..1128: note = a matured form of a standard esterase (quintuple mutant)
  source 1..1128: mol_type = other DNA
gtggatgcacagacgattgcccctggattcgaatcagtcgccgaactctttggccgtttcctgagcgaagaccgggaatattcagcccagctcgcggcctaccaccgcggagtcaaggtattggacatcagcggtgggccgcaccgccgcccggattccgtgaccggtgttttctcctgctccaagggagtatccgggctggtcatcgcacttttggtccaggacggcttcctcgacctcgacgccgaagtggtcaagtactggccggaattcggcgccgaaggaaaggccacgattaccgtggcccagctgctctcccaccaggccgggcttctgggagtcgaaggcggactcaccctcgcggaatacaacaactccgaactggccgccgccaagctcgcgcagatgcggccgctgtggaagcccgggaccgccttcgggtaccacgccctgaccatcggcgtcttcatggaggagctttgccgccggatcaccgggtccacgctccaggaaatctacgaacagcggatccgctcggtcacgggcgcccacttcttcctgggactgcctgagtccgaggaaccccgctatgccaccctccgttgggctgcagacccctcccagccgtggattgatcccgccagccatttcggcctttcctttgactcggccgtgggggacatccttgacctgcccaacctccgcgaggtccgcgcagccggcctgagttcagccgccggagtcgccagcgcggaaggcatggcccgcgtctacgctgcggcactcaccggacttgccgccaacggcgaccgagccgccgtcgcgcccctcctcagcgaagagaccatccaaaccgtcacggccgagcaggtcttcggcatcgaccgggtgctcggcgagacgagctgctttgggacagtgttcatgaaatcgcatgcacgctcgccttatggcagctaccgggcgttcgggcacgtcggcgggagcgcatctttggggttcgctgaccctgtgtatgaactcgccttcgggtacgtgccgcaacaggccgagccgggcggagcgggatgccgcaaccttgagctgagcgccgccgtgcggaaggcagtcaccgaactggctcagtag

SEQ ID NO: 14 - DNA, 1152 bp, synthetic construct
  misc_feature 1..1152: note = a full-length form of a standard esterase (quintuple mutant)
  source 1..1152: mol_type = other DNA
atgaccatgattacgccaagcttggtggatgcacagacgattgcccctggattcgaatcagtcgccgaactctttggccgtttcctgagcgaagaccgggaatattcagcccagctcgcggcctaccaccgcggagtcaaggtattggacatcagcggtgggccgcaccgccgcccggattccgtgaccggtgttttctcctgctccaagggagtatccgggctggtcatcgcacttttggtccaggacggcttcctcgacctcgacgccgaagtggtcaagtactggccggaattcggcgccgaaggaaaggccacgattaccgtggcccagctgctctcccaccaggccgggcttctgggagtcgaaggcggactcaccctcgcggaatacaacaactccgaactggccgccgccaagctcgcgcagatgcggccgctgtggaagcccgggaccgccttcgggtaccacgccctgaccatcggcgtcttcatggaggagctttgccgccggatcaccgggtccacgctccaggaaatctacgaacagcggatccgctcggtcacgggcgcccacttcttcctgggactgcctgagtccgaggaaccccgctatgccaccctccgttgggctgcagacccctcccagccgtggattgatcccgccagccatttcggcctttcctttgactcggccgtgggggacatccttgacctgcccaacctccgcgaggtccgcgcagccggcctgagttcagccgccggagtcgccagcgcggaaggcatggcccgcgtctacgctgcggcactcaccggacttgccgccaacggcgaccgagccgccgtcgcgcccctcctcagcgaagagaccatccaaaccgtcacggccgagcaggtcttcggcatcgaccgggtgctcggcgagacgagctgctttgggacagtgttcatgaaatcgcatgcacgctcgccttatggcagctaccgggcgttcgggcacgtcggcgggagcgcatctttggggttcgctgaccctgtgtatgaactcgccttcgggtacgtgccgcaacaggccgagccgggcggagcgggatgccgcaaccttgagctgagcgccgccgtgcggaaggcagtcaccgaactggctcagtag

SEQ ID NO: 15 - DNA, 1128 bp, Arthrobacter globiformis
  source 1..1128: mol_type = other DNA
gtggatgcacagacgattgcccctggattcgaatcagtcgccgaactctttggccgtttcctgagcgaagaccgggaatattcagcccagctcgcggcctaccaccgcggagtcaaggtattggacatcagcggtgggccgcaccgccgcccggattccgtgaccggtgttttctcctgctccaagggagtatccgggctggtcatcgcacttttggtccaggacggcttcctcgacctcgacgccgaagtggtcaagtactggccggaattcggcgccgaaggaaaggccacgattaccgtggcccagctgctctcccaccaggccgggcttctgggagtcgaaggcggactcaccctcgcggaatacaacaactccgaactggccgccgccaagctcgcgcagatgcggccgctgtggaagcccgggaccgccttcgggtaccacgccctgaccatcggcgtcttcatggaggagctttgccgccggatcaccgggtccacgctccaggaaatctacgaacagcggatccgctcggtcacgggcgcccacttcttcctgggactgcctgagtccgaggaaccccgctatgccaccctccgttgggctgcagacccctcccagccgtggattgatcccgccagccatttcggcctttccgcaaactcggccgtgggggacatccttgacctgcccaacctccgcgaggtccgcgcagccggcctgagttcagccgccggagtcgccagcgcggaaggcatggcccgcgtctacgctgcggcactcaccggacttgccgccaacggcgaccgagccgccgtcgcgcccctcctcagcgaagagaccatccaaaccgtcacggccgagcaggtcttcggcatcgaccgggtgttcggcgagacgagctgctttgggacagtgttcatgaaatcgcatgcacgctcgccttatggcagctaccgggcgttcgggcacgacggcgccagcgcatctttggggttcgctgaccctgtgtatgaactcgccttcgggtacgtgccgcaacaggccgagccgggcggagcgggatgccgcaaccttgagctgagcgccgccgtgcggaaggcagtcaccgaactggctcagtag

SEQ ID NO: 16 - DNA, 1152 bp, Arthrobacter globiformis
  source 1..1152: mol_type = other DNA
atgaccatgattacgccaagcttggtggatgcacagacgattgcccctggattcgaatcagtcgccgaactctttggccgtttcctgagcgaagaccgggaatattcagcccagctcgcggcctaccaccgcggagtcaaggtattggacatcagcggtgggccgcaccgccgcccggattccgtgaccggtgttttctcctgctccaagggagtatccgggctggtcatcgcacttttggtccaggacggcttcctcgacctcgacgccgaagtggtcaagtactggccggaattcggcgccgaaggaaaggccacgattaccgtggcccagctgctctcccaccaggccgggcttctgggagtcgaaggcggactcaccctcgcggaatacaacaactccgaactggccgccgccaagctcgcgcagatgcggccgctgtggaagcccgggaccgccttcgggtaccacgccctgaccatcggcgtcttcatggaggagctttgccgccggatcaccgggtccacgctccaggaaatctacgaacagcggatccgctcggtcacgggcgcccacttcttcctgggactgcctgagtccgaggaaccccgctatgccaccctccgttgggctgcagacccctcccagccgtggattgatcccgccagccatttcggcctttccgcaaactcggccgtgggggacatccttgacctgcccaacctccgcgaggtccgcgcagccggcctgagttcagccgccggagtcgccagcgcggaaggcatggcccgcgtctacgctgcggcactcaccggacttgccgccaacggcgaccgagccgccgtcgcgcccctcctcagcgaagagaccatccaaaccgtcacggccgagcaggtcttcggcatcgaccgggtgttcggcgagacgagctgctttgggacagtgttcatgaaatcgcatgcacgctcgccttatggcagctaccgggcgttcgggcacgacggcgccagcgcatctttggggttcgctgaccctgtgtatgaactcgccttcgggtacgtgccgcaacaggccgagccgggcggagcgggatgccgcaaccttgagctgagcgccgccgtgcggaaggcagtcaccgaactggctcagtag

SEQ ID NO: 17 - DNA, 1128 bp, synthetic construct
  misc_feature 1..1128: note = L151F mutant of SEQ ID NO:1
  source 1..1128: mol_type = other DNA
gtggatgcacagacgattgcccctggattcgaatcagtcgccgaactctttggccgtttcctgagcgaagaccgggaatattcagcccagctcgcggcctaccaccgcggagtcaaggtattggacatcagcggtgggccgcaccgccgcccggattccgtgaccggtgttttctcctgctccaagggagtatccgggctggtcatcgcacttttggtccaggacggcttcctcgacctcgacgccgaagtggtcaagtactggccggaattcggcgccgaaggaaaggccacgattaccgtggcccagctgctctcccaccaggccgggcttctgggagtcgaaggcggactcaccctcgcggaatacaacaactccgaactggccgccgccaagctcgcgcagatgcggccgctgtggaagcccgggaccgccttcgggtaccacgcctttaccatcggcgtcttcatggaggagctttgccgccggatcaccgggtccacgctccaggaaatctacgaacagcggatccgctcggtcacgggcgcccacttcttcctgggactgcctgagtccgaggaaccccgctatgccaccctccgttgggctgcagacccctcccagccgtggattgatcccgccagccatttcggcctttcctttgactcggccgtgggggacatccttgacctgcccaacctccgcgaggtccgcgcagccggcctgagttcagccgccggagtcgccagcgcggaaggcatggcccgcgtctacgctgcggcactcaccggacttgccgccaacggcgaccgagccgccgtcgcgcccctcctcagcgaagagaccatccaaaccgtcacggccgagcaggtcttcggcatcgaccgggtgctcggcgagacgagctgctttgggacagtgttcatgaaatcgcatgcacgctcgccttatggcagctaccgggcgttcgggcacgtcggcgggagcgcatctttggggttcgctgaccctgtgtatgaactcgccttcgggtacgtgccgcaacaggccgagccgggcggagcgggatgccgcaaccttgagctgagcgccgccgtgcggaaggcagtcaccgaactggctcagtag

SEQ ID NO: 18 - DNA, 1128 bp, synthetic construct
  misc_feature 1..1128: note = L242M mutant of SEQ ID NO:1
  source 1..1128: mol_type = other DNA
gtggatgcacagacgattgcccctggattcgaatcagtcgccgaactctttggccgtttcctgagcgaagaccgggaatattcagcccagctcgcggcctaccaccgcggagtcaaggtattggacatcagcggtgggccgcaccgccgcccggattccgtgaccggtgttttctcctgctccaagggagtatccgggctggtcatcgcacttttggtccaggacggcttcctcgacctcgacgccgaagtggtcaagtactggccggaattcggcgccgaaggaaaggccacgattaccgtggcccagctgctctcccaccaggccgggcttctgggagtcgaaggcggactcaccctcgcggaatacaacaactccgaactggccgccgccaagctcgcgcagatgcggccgctgtggaagcccgggaccgccttcgggtaccacgccctgaccatcggcgtcttcatggaggagctttgccgccggatcaccgggtccacgctccaggaaatctacgaacagcggatccgctcggtcacgggcgcccacttcttcctgggactgcctgagtccgaggaaccccgctatgccaccctccgttgggctgcagacccctcccagccgtggattgatcccgccagccatttcggcctttcctttgactcggccgtgggggacatccttgacctgcccaacctccgcgaggtccgcgcagccggcatgagttcagccgccggagtcgccagcgcggaaggcatggcccgcgtctacgctgcggcactcaccggacttgccgccaacggcgaccgagccgccgtcgcgcccctcctcagcgaagagaccatccaaaccgtcacggccgagcaggtcttcggcatcgaccgggtgctcggcgagacgagctgctttgggacagtgttcatgaaatcgcatgcacgctcgccttatggcagctaccgggcgttcgggcacgtcggcgggagcgcatctttggggttcgctgaccctgtgtatgaactcgccttcgggtacgtgccgcaacaggccgagccgggcggagcgggatgccgcaaccttgagctgagcgccgccgtgcggaaggcagtcaccgaactggctcagtag

SEQ ID NO: 19 - DNA, 1128 bp, synthetic construct
  misc_feature 1..1128: note = S329N mutant of SEQ ID NO:1
  source 1..1128: mol_type = other DNA
gtggatgcacagacgattgcccctggattcgaatcagtcgccgaactctttggccgtttcctgagcgaagaccgggaatattcagcccagctcgcggcctaccaccgcggagtcaaggtattggacatcagcggtgggccgcaccgccgcccggattccgtgaccggtgttttctcctgctccaagggagtatccgggctggtcatcgcacttttggtccaggacggcttcctcgacctcgacgccgaagtggtcaagtactggccggaattcggcgccgaaggaaaggccacgattaccgtggcccagctgctctcccaccaggccgggcttctgggagtcgaaggcggactcaccctcgcggaatacaacaactccgaactggccgccgccaagctcgcgcagatgcggccgctgtggaagcccgggaccgccttcgggtaccacgccctgaccatcggcgtcttcatggaggagctttgccgccggatcaccgggtccacgctccaggaaatctacgaacagcggatccgctcggtcacgggcgcccacttcttcctgggactgcctgagtccgaggaaccccgctatgccaccctccgttgggctgcagacccctcccagccgtggattgatcccgccagccatttcggcctttcctttgactcggccgtgggggacatccttgacctgcccaacctccgcgaggtccgcgcagccggcctgagttcagccgccggagtcgccagcgcggaaggcatggcccgcgtctacgctgcggcactcaccggacttgccgccaacggcgaccgagccgccgtcgcgcccctcctcagcgaagagaccatccaaaccgtcacggccgagcaggtcttcggcatcgaccgggtgctcggcgagacgagctgctttgggacagtgttcatgaaatcgcatgcacgctcgccttatggcagctaccgggcgttcgggcacgtcggcgggaatgcatctttggggttcgctgaccctgtgtatgaactcgccttcgggtacgtgccgcaacaggccgagccgggcggagcgggatgccgcaaccttgagctgagcgccgccgtgcggaaggcagtcaccgaactggctcagtag

SEQ ID NO: 20 - DNA, 1128 bp, synthetic construct
  misc_feature 1..1128: note = L200F mutant of SEQ ID NO:1
  source 1..1128: mol_type = other DNA
gtggatgcacagacgattgcccctggattcgaatcagtcgccgaactctttggccgtttcctgagcgaagaccgggaatattcagcccagctcgcggcctaccaccgcggagtcaaggtattggacatcagcggtgggccgcaccgccgcccggattccgtgaccggtgttttctcctgctccaagggagtatccgggctggtcatcgcacttttggtccaggacggcttcctcgacctcgacgccgaagtggtcaagtactggccggaattcggcgccgaaggaaaggccacgattaccgtggcccagctgctctcccaccaggccgggcttctgggagtcgaaggcggactcaccctcgcggaatacaacaactccgaactggccgccgccaagctcgcgcagatgcggccgctgtggaagcccgggaccgccttcgggtaccacgccctgaccatcggcgtcttcatggaggagctttgccgccggatcaccgggtccacgctccaggaaatctacgaacagcggatccgctcggtcacgggcgcccacttcttcctgggactgcctgagtccgaggaaccccgctatgccacctttcgttgggctgcagacccctcccagccgtggattgatcccgccagccatttcggcctttcctttgactcggccgtgggggacatccttgacctgcccaacctccgcgaggtccgcgcagccggcctgagttcagccgccggagtcgccagcgcggaaggcatggcccgcgtctacgctgcggcactcaccggacttgccgccaacggcgaccgagccgccgtcgcgcccctcctcagcgaagagaccatccaaaccgtcacggccgagcaggtcttcggcatcgaccgggtgctcggcgagacgagctgctttgggacagtgttcatgaaatcgcatgcacgctcgccttatggcagctaccgggcgttcgggcacgtcggcgggagcgcatctttggggttcgctgaccctgtgtatgaactcgccttcgggtacgtgccgcaacaggccgagccgggcggagcgggatgccgcaaccttgagctgagcgccgccgtgcggaaggcagtcaccgaactggctcagtag

SEQ ID NO: 21 - DNA, 1128 bp, synthetic construct
  misc_feature 1..1128: note = L151F/L242M mutant of SEQ ID NO:1
  source 1..1128: mol_type = other DNA
gtggatgcacagacgattgcccctggattcgaatcagtcgccgaactctttggccgtttcctgagcgaagaccgggaatattcagcccagctcgcggcctaccaccgcggagtcaaggtattggacatcagcggtgggccgcaccgccgcccggattccgtgaccggtgttttctcctgctccaagggagtatccgggctggtcatcgcacttttggtccaggacggcttcctcgacctcgacgccgaagtggtcaagtactggccggaattcggcgccgaaggaaaggccacgattaccgtggcccagctgctctcccaccaggccgggcttctgggagtcgaaggcggactcaccctcgcggaatacaacaactccgaactggccgccgccaagctcgcgcagatgcggccgctgtggaagcccgggaccgccttcgggtaccacgcctttaccatcggcgtcttcatggaggagctttgccgccggatcaccgggtccacgctccaggaaatctacgaacagcggatccgctcggtcacgggcgcccacttcttcctgggactgcctgagtccgaggaaccccgctatgccaccctccgttgggctgcagacccctcccagccgtggattgatcccgccagccatttcggcctttcctttgactcggccgtgggggacatccttgacctgcccaacctccgcgaggtccgcgcagccggcatgagttcagccgccggagtcgccagcgcggaaggcatggcccgcgtctacgctgcggcactcaccggacttgccgccaacggcgaccgagccgccgtcgcgcccctcctcagcgaagagaccatccaaaccgtcacggccgagcaggtcttcggcatcgaccgggtgctcggcgagacgagctgctttgggacagtgttcatgaaatcgcatgcacgctcgccttatggcagctaccgggcgttcgggcacgtcggcgggagcgcatctttggggttcgctgaccctgtgtatgaactcgccttcgggtacgtgccgcaacaggccgagccgggcggagcgggatgccgcaaccttgagctgagcgccgccgtgcggaaggcagtcaccgaactggctcagtag

SEQ ID NO: 22 - DNA, 1128 bp, synthetic construct
  misc_feature 1..1128: note = L151F/L242M/S329N mutant of SEQ ID NO:1
  source 1..1128: mol_type = other DNA
gtggatgcacagacgattgcccctggattcgaatcagtcgccgaactctttggccgtttcctgagcgaagaccgggaatattcagcccagctcgcggcctaccaccgcggagtcaaggtattggacatcagcggtgggccgcaccgccgcccggattccgtgaccggtgttttctcctgctccaagggagtatccgggctggtcatcgcacttttggtccaggacggcttcctcgacctcgacgccgaagtggtcaagtactggccggaattcggcgccgaaggaaaggccacgattaccgtggcccagctgctctcccaccaggccgggcttctgggagtcgaaggcggactcaccctcgcggaatacaacaactccgaactggccgccgccaagctcgcgcagatgcggccgctgtggaagcccgggaccgccttcgggtaccacgcctttaccatcggcgtcttcatggaggagctttgccgccggatcaccgggtccacgctccaggaaatctacgaacagcggatccgctcggtcacgggcgcccacttcttcctgggactgcctgagtccgaggaaccccgctatgccaccctccgttgggctgcagacccctcccagccgtggattgatcccgccagccatttcggcctttcctttgactcggccgtgggggacatccttgacctgcccaacctccgcgaggtccgcgcagccggcatgagttcagccgccggagtcgccagcgcggaaggcatggcccgcgtctacgctgcggcactcaccggacttgccgccaacggcgaccgagccgccgtcgcgcccctcctcagcgaagagaccatccaaaccgtcacggccgagcaggtcttcggcatcgaccgggtgctcggcgagacgagctgctttgggacagtgttcatgaaatcgcatgcacgctcgccttatggcagctaccgggcgttcgggcacgtcggcgggaatgcatctttggggttcgctgaccctgtgtatgaactcgccttcgggtacgtgccgcaacaggccgagccgggcggagcgggatgccgcaaccttgagctgagcgccgccgtgcggaaggcagtcaccgaactggctcagtag

SEQ ID NO: 23 - DNA, 1128 bp, synthetic construct
  misc_feature 1..1128: note = L151F/L242M/L200F mutant of SEQ ID NO:1
  source 1..1128: mol_type = other DNA
gtggatgcacagacgattgcccctggattcgaatcagtcgccgaactctttggccgtttcctgagcgaagaccgggaatattcagcccagctcgcggcctaccaccgcggagtcaaggtattggacatcagcggtgggccgcaccgccgcccggattccgtgaccggtgttttctcctgctccaagggagtatccgggctggtcatcgcacttttggtccaggacggcttcctcgacctcgacgccgaagtggtcaagtactggccggaattcggcgccgaaggaaaggccacgattaccgtggcccagctgctctcccaccaggccgggcttctgggagtcgaaggcggactcaccctcgcggaatacaacaactccgaactggccgccgccaagctcgcgcagatgcggccgctgtggaagcccgggaccgccttcgggtaccacgcctttaccatcggcgtcttcatggaggagctttgccgccggatcaccgggtccacgctccaggaaatctacgaacagcggatccgctcggtcacgggcgcccacttcttcctgggactgcctgagtccgaggaaccccgctatgccacctttcgttgggctgcagacccctcccagccgtggattgatcccgccagccatttcggcctttcctttgactcggccgtgggggacatccttgacctgcccaacctccgcgaggtccgcgcagccggcatgagttcagccgccggagtcgccagcgcggaaggcatggcccgcgtctacgctgcggcactcaccggacttgccgccaacggcgaccgagccgccgtcgcgcccctcctcagcgaagagaccatccaaaccgtcacggccgagcaggtcttcggcatcgaccgggtgctcggcgagacgagctgctttgggacagtgttcatgaaatcgcatgcacgctcgccttatggcagctaccgggcgttcgggcacgtcggcgggagcgcatctttggggttcgctgaccctgtgtatgaactcgccttcgggtacgtgccgcaacaggccgagccgggcggagcgggatgccgcaaccttgagctgagcgccgccgtgcggaaggcagtcaccgaactggctcagtag

SEQ ID NO: 24 - DNA, 1128 bp, synthetic construct
  misc_feature 1..1128: note = L151F/L242M/L200F/S329N mutant of SEQ ID NO:1
  source 1..1128: mol_type = other DNA
gtggatgcacagacgattgcccctggattcgaatcagtcgccgaactctttggccgtttcctgagcgaagaccgggaatattcagcccagctcgcggcctaccaccgcggagtcaaggtattggacatcagcggtgggccgcaccgccgcccggattccgtgaccggtgttttctcctgctccaagggagtatccgggctggtcatcgcacttttggtccaggacggcttcctcgacctcgacgccgaagtggtcaagtactggccggaattcggcgccgaaggaaaggccacgattaccgtggcccagctgctctcccaccaggccgggcttctgggagtcgaaggcggactcaccctcgcggaatacaacaactccgaactggccgccgccaagctcgcgcagatgcggccgctgtggaagcccgggaccgccttcgggtaccacgcctttaccatcggcgtcttcatggaggagctttgccgccggatcaccgggtccacgctccaggaaatctacgaacagcggatccgctcggtcacgggcgcccacttcttcctgggactgcctgagtccgaggaaccccgctatgccacctttcgttgggctgcagacccctcccagccgtggattgatcccgccagccatttcggcctttcctttgactcggccgtgggggacatccttgacctgcccaacctccgcgaggtccgcgcagccggcatgagttcagccgccggagtcgccagcgcggaaggcatggcccgcgtctacgctgcggcactcaccggacttgccgccaacggcgaccgagccgccgtcgcgcccctcctcagcgaagagaccatccaaaccgtcacggccgagcaggtcttcggcatcgaccgggtgctcggcgagacgagctgctttgggacagtgttcatgaaatcgcatgcacgctcgccttatggcagctaccgggcgttcgggcacgtcggcgggaatgcatctttggggttcgctgaccctgtgtatgaactcgccttcgggtacgtgccgcaacaggccgagccgggcggagcgggatgccgcaaccttgagctgagcgccgccgtgcggaaggcagtcaccgaactggctcagtag

SEQ ID NO: 25 - DNA, 27 bp, synthetic construct
  misc_feature 1..27: note = Fw primer for preparation of 151 mutant liabrary
  misc_feature 1..2: note = n is a, c, g, or t
  source 1..27: mol_type = other DNA
nnkaccatcggcgtcttcatggaggag

SEQ ID NO: 26 - DNA, 24 bp, synthetic construct
  misc_feature 1..24: note = Rv primer for preparation of 151 mutant liabrary
  source 1..24: mol_type = other DNA
ggcgtggtacccgaaggcggtccc

SEQ ID NO: 27 - DNA, 24 bp, synthetic construct
  misc_feature 1..24: note = Fw primer for preparation of 242 mutant liabrary
  misc_feature 1..2: note = n is a, c, g, or t
  source 1..24: mol_type = other DNA
nnkagttcagccgccggagtcgcc

SEQ ID NO: 28 - DNA, 25 bp, synthetic construct
  misc_feature 1..25: note = Rv primer for preparation of 242 mutant liabrary
  source 1..25: mol_type = other DNA
gccggctgcgcggacctcgcggagg

SEQ ID NO: 29 - DNA, 19 bp, synthetic construct
  misc_feature 1..19: note = Fw primer for random mutation
  source 1..19: mol_type = other DNA
atatgaccatgattacgcc

SEQ ID NO: 30 - DNA, 19 bp, synthetic construct
  misc_feature 1..19: note = Rv primer for random mutation
  source 1..19: mol_type = other DNA
tggtgctcgagctactgag